European Patent Application EP 4 722 380 A1, published April 8, 2026. Title: 甲醛重交联在CUT&Tag技术建库中的应用. Applicant: 上海近岸科技有限公司. The sequence listing filed with the application follows.

SEQUENCE LISTING (12 sequences)

SEQ ID NO: 1 - DNA, 52 bp, synthetic construct
  source 1..52: mol_type = other DNA
aatgatacggcgaccaccgagatctacactagatcgctcgtcggcagcgtca

SEQ ID NO: 2 - DNA, 52 bp, synthetic construct
  source 1..52: mol_type = other DNA
aatgatacggcgaccaccgagatctacacctctctattcgtcggcagcgtca

SEQ ID NO: 3 - DNA, 52 bp, synthetic construct
  source 1..52: mol_type = other DNA
aatgatacggcgaccaccgagatctacactatcctcttcgtcggcagcgtca

SEQ ID NO: 4 - DNA, 52 bp, synthetic construct
  source 1..52: mol_type = other DNA
aatgatacggcgaccaccgagatctacacagagtagatcgtcggcagcgtca

SEQ ID NO: 5 - DNA, 52 bp, synthetic construct
  source 1..52: mol_type = other DNA
aatgatacggcgaccaccgagatctacacgtaaggagtcgtcggcagcgtca

SEQ ID NO: 6 - DNA, 47 bp, synthetic construct
  source 1..47: mol_type = other DNA
caagcagaagacggcatacgagattcgccttagtctcgtgggctcgg

SEQ ID NO: 7 - DNA, 47 bp, synthetic construct
  source 1..47: mol_type = other DNA
caagcagaagacggcatacgagatctagtacggtctcgtgggctcgg

SEQ ID NO: 8 - DNA, 47 bp, synthetic construct
  source 1..47: mol_type = other DNA
caagcagaagacggcatacgagatttctgcctgtctcgtgggctcgg

SEQ ID NO: 9 - DNA, 47 bp, synthetic construct
  source 1..47: mol_type = other DNA
caagcagaagacggcatacgagatgctcaggagtctcgtgggctcgg

SEQ ID NO: 10 - DNA, 47 bp, synthetic construct
  source 1..47: mol_type = other DNA
caagcagaagacggcatacgagataggagtccgtctcgtgggctcgg

SEQ ID NO: 11 - DNA, 29 bp, synthetic construct
  source 1..29: mol_type = other DNA
aatgatacggcgaccaccgagatctacac

SEQ ID NO: 12 - DNA, 24 bp, synthetic construct
  source 1..24: mol_type = other DNA
caagcagaagacggcatacgagat